European Patent Application EP 4 541 887 A2, published April 23, 2025. Title: COMPOSITIONS AND METHODS FOR PREPARING FACTOR XA AND DERIVATIVES. Applicant: ALEXION PHARMACEUTICALS, INC. Application EP. The sequence listing filed with the application follows.

SEQUENCE LISTING (49 sequences)

SEQ ID NO: 1 - protein, 488 aa, Homo sapiens
MGRPLHLVLLSASLAGLLLLGESLFIRREQANNILARVTRANSFLEEMKKGHLERECMEETCSYEEAREVFEDSDKTNEFWNKYKDGDQCETSPCQNQGKCKDGLGEYTCTCLEGFEGKNCELFTRKLCSLDNGDCDQFCHEEQNSVVCSCARGYTLADNGKACIPTGPYPCGKQTLERRKRSVAQATSSSGEAPDSITWKPYDAADLDPTENPFDLLDFNQTQPERGDNNLTRIVGGQECKDGECPWQALLINEENEGFCGGTILSEFYILTAAHCLYQAKRFKVRVGDRNTEQEEGGEAVHEVEVVIKHNRFTKETYDFDIAVLRLKTPITFRMNVAPACLPERDWAESTLMTQKTGIVSGFGRTHEKGRQSTRLKMLEVPYVDRNSCKLSSSFIITQNMFCAGYDTKQEDACQGDSGGPHVTRFKDTYFVTGIVSWGEGCARKGKYGIYTKVTAFLKWIDRSMKTRGLPKAKSHAPEVITSSPLK

SEQ ID NO: 2 - protein, 448 aa, Homo sapiens [sequence omitted]

SEQ ID NO: 3 - protein, 393 aa, synthetic construct
  REGION 1..393: note = Description of Artificial Sequence: Synthetic polypeptide
ANSFLEEMKKGHLERECMEETCSYEEAREVFEDSDKTNEFWNKYKDGDQCETSPCQNQGKCKDGLGEYTCTCLEGFEGKNCELFTRKLCSLDNGDCDQFCHEEQNSVVCSCARGYTLADNGKACIPTGPYPCGKQTLERIVGGQECKDGECPWQALLINEENEGFCGGTILSEFYILTAAHCLYQAKRFKVRVGDRNTEQEEGGEAVHEVEVVIKHNRFTKETYDFDIAVLRLKTPITFRMNVAPACLPERDWAESTLMTQKTGIVSGFGRTHEKGRQSTRLKMLEVPYVDRNSCKLSSSFIITQNMFCAGYDTKQEDACQGDSGGPHVTRFKDTYFVTGIVSWGEGCARKGKYGIYTKVTAFLKWIDRSMKTRGLPKAKSHAPEVITSSPLK

SEQ ID NO: 4 - protein, 365 aa, synthetic construct
  REGION 1..365: note = Description of Artificial Sequence: Synthetic polypeptide
ANSFLFWNKYKDGDQCETSPCQNQGKCKDGLGEYTCTCLEGFEGKNCELFTRKLCSLDNGDCDQFCHEEQNSVVCSCARGYTLADNGKACIPTGPYPCGKQTLERRKRRKRIVGGQECKDGECPWQALLINEENEGFCGGTILSEFYILTAAHCLYQAKRFKVRVGDRNTEQEEGGEAVHEVEVVIKHNRFTKETYDFDIAVLRLKTPITFRMNVAPACLPERDWAESTLMTQKTGIVSGFGRTHEKGRQSTRLKMLEVPYVDRNSCKLSSSFIITQNMFCAGYDTKQEDACQGDAGGPHVTRFKDTYFVTGIVSWGEGCARKGKYGIYTKVTAFLKWIDRSMKTRGLPKAKSHAPEVITSSPLK

SEQ ID NO: 5 - protein, 359 aa, synthetic construct
  REGION 1..359: note = Description of Artificial Sequence: Synthetic polypeptide
ANSFLFWNKYKDGDQCETSPCQNQGKCKDGLGEYTCTCLEGFEGKNCELFTRKLCSLDNGDCDQFCHEEQNSVVCSCARGYTLADNGKACIPTGPYPCGKQTLERIVGGQECKDGECPWQALLINEENEGFCGGTILSEFYILTAAHCLYQAKRFKVRVGDRNTEQEEGGEAVHEVEVVIKHNRFTKETYDFDIAVLRLKTPITFRMNVAPACLPERDWAESTLMTQKTGIVSGFGRTHEKGRQSTRLKMLEVPYVDRNSCKLSSSFIITQNMFCAGYDTKQEDACQGDAGGPHVTRFKDTYFVTGIVSWGEGCARKGKYGIYTKVTAFLKWIDRSMKTRGLPKAKSHAPEVITSSPLK

SEQ ID NO: 6 - protein, 105 aa, synthetic construct
  REGION 1..105: note = Description of Artificial Sequence: Synthetic polypeptide
ANSFLFWNKYKDGDQCETSPCQNQGKCKDGLGEYTCTCLEGFEGKNCELFTRKLCSLDNGDCDQFCHEEQNSVVCSCARGYTLADNGKACIPTGPYPCGKQTLER

SEQ ID NO: 7 - protein, 6 aa, synthetic construct
  REGION 1..6: note = Description of Artificial Sequence: Synthetic peptide
RKRRKR

SEQ ID NO: 8 - protein, 254 aa, synthetic construct
  REGION 1..254: note = Description of Artificial Sequence: Synthetic polypeptide
IVGGQECKDGECPWQALLINEENEGFCGGTILSEFYILTAAHCLYQAKRFKVRVGDRNTEQEEGGEAVHEVEVVIKHNRFTKETYDFDIAVLRLKTPITFRMNVAPACLPERDWAESTLMTQKTGIVSGFGRTHEKGRQSTRLKMLEVPYVDRNSCKLSSSFIITQNMFCAGYDTKQEDACQGDAGGPHVTRFKDTYFVTGIVSWGEGCARKGKYGIYTKVTAFLKWIDRSMKTRGLPKAKSHAPEVITSSPLK

SEQ ID NO: 9 - protein, 234 aa, synthetic construct
  REGION 1..234: note = Description of Artificial Sequence: Synthetic polypeptide
IVGGQECKDGECPWQALLINEENEGFCGGTILSEFYILTAAHCLYQAKRFKVRVGDRNTEQEEGGEAVHEVEVVIKHNRFTKETYDFDIAVLRLKTPITFRMNVAPACLPERDWAESTLMTQKTGIVSGFGRTHEKGRQSTRLKMLEVPYVDRNSCKLSSSFIITQNMFCAGYDTKQEDACQGDAGGPHVTRFKDTYFVTGIVSWGEGCARKGKYGIYTKVTAFLKWIDRSMKT

SEQ ID NO: 10 - protein, 241 aa, synthetic construct
  REGION 1..241: note = Description of Artificial Sequence: Synthetic polypeptide
IVGGQECKDGECPWQALLINEENEGFCGGTILSEFYILTAAHCLYQAKRFKVRVGDRNTEQEEGGEAVHEVEVVIKHNRFTKETYDFDIAVLRLKTPITFRMNVAPACLPERDWAESTLMTQKTGIVSGFGRTHEKGRQSTRLKMLEVPYVDRNSCKLSSSFIITQNMFCAGYDTKQEDACQGDAGGPHVTRFKDTYFVTGIVSWGEGCARKGKYGIYTKVTAFLKWIDRSMKTRGLPKAK

SEQ ID NO: 11 - protein, 239 aa, synthetic construct
  REGION 1..239: note = Description of Artificial Sequence: Synthetic polypeptide
IVGGQECKDGECPWQALLINEENEGFCGGTILSEFYILTAAHCLYQAKRFKVRVGDRNTEQEEGGEAVHEVEVVIKHNRFTKETYDFDIAVLRLKTPITFRMNVAPACLPERDWAESTLMTQKTGIVSGFGRTHEKGRQSTRLKMLEVPYVDRNSCKLSSSFIITQNMFCAGYDTKQEDACQGDAGGPHVTRFKDTYFVTGIVSWGEGCARKGKYGIYTKVTAFLKWIDRSMKTRGLPK

SEQ ID NO: 12 - protein, 52 aa, synthetic construct
  REGION 1..52: note = Description of Artificial Sequence: Synthetic polypeptide
SVAQATSSSGEAPDSITWKPYDAADLDPTENPFDLLDFNQTQPERGDNNLTR

SEQ ID NO: 13 - protein, 94 aa, synthetic construct
  REGION 1..94: note = Description of Artificial Sequence: Synthetic polypeptide
DGDQCETSPCQNQGKCKDGLGEYTCTCLEGFEGKNCELFTRKLCSLDNGDCDQFCHEEQNSVVCSCARGYTLADNGKACIPTGPYPCGKQTLER

SEQ ID NO: 14 - protein, 31 aa, synthetic construct
  REGION 1..31: note = Description of Artificial Sequence: Synthetic polypeptide
SSGGSGGSGGSGGSGGSGGSGGSGGSGGSGS

SEQ ID NO: 15 - protein, 585 aa, Homo sapiens
DAHKSEVAHRFKDLGEENFKALVLIAFAQYLQQSPFEDHVKLVNEVTEFAKTCVADESAENCDKSLHTLFGDKLCTVATLRETYGEMADCCAKQEPERNECFLQHKDDNPNLPRLVRPEVDVMCTAFHDNEETFLKKYLYEIARRHPYFYAPELLFFAKRYKAAFTECCQAADKAACLLPKLDELRDEGKASSAKQRLKCASLQKFGERAFKAWAVARLSQRFPKAEFAEVSKLVTDLTKVHTECCHGDLLECADDRADLAKYICENQDSISSKLKECCEKPLLEKSHCIAEVENDEMPADLPSLAADFVESKDVCKNYAEAKDVFLGMFLYEYARRHPDYSVVLLLRLAKTYETTLEKCCAAADPHECYAKVFDEFKPLVEEPQNLIKQNCELFEQLGEYKFQNALLVRYTKKVPQVSTPTLVEVSRNLGKVGSKCCKHPEAKRMPCAEDYLSVVLNQLCVLHEKTPVSDRVTKCCTESLVNRRPCFSALEVDETYVPKEFNAETFTFHADICTLSEKERQIKKQTALVELVKHKPKATKEQLKAVMDDFAAFVEKCCKADDKETCFAEEGKKLVAASQAALGL

SEQ ID NO: 16 - protein, 291 aa, synthetic construct
  REGION 1..291: note = Description of Artificial Sequence: Synthetic polypeptide
IVGGQECKDGECPWQALLINEENEGFCGGTILSEFYILTAAHCLYQAKRFKVRVGDRNTEQEEGGEAVHEVEVVIKHNRFTKETYDFDIAVLRLKTPITFRMNVAPACLPERDWAESTLMTQKTGIVSGFGRTHEKGRQSTRLKMLEVPYVDRNSCKLSSSFIITQNMFCAGYDTKQEDACQGDAGGPHVTRFKDTYFVTGIVSWGEGCARKGKYGIYTKVTAFLKWIDRSMKTRGLPKSVAQATSSSGEAPDSITWKPYDAADLDPTENPFDLLDFNQTQPERGDNNLTR

SEQ ID NO: 17 - protein, 322 aa, synthetic construct
  REGION 1..322: note = Description of Artificial Sequence: Synthetic polypeptide
IVGGQECKDGECPWQALLINEENEGFCGGTILSEFYILTAAHCLYQAKRFKVRVGDRNTEQEEGGEAVHEVEVVIKHNRFTKETYDFDIAVLRLKTPITFRMNVAPACLPERDWAESTLMTQKTGIVSGFGRTHEKGRQSTRLKMLEVPYVDRNSCKLSSSFIITQNMFCAGYDTKQEDACQGDAGGPHVTRFKDTYFVTGIVSWGEGCARKGKYGIYTKVTAFLKWIDRSMKTRGLPKSSGGSGGSGGSGGSGGSGGSGGSGGSGGSGSSVAQATSSSGEAPDSITWKPYDAADLDPTENPFDLLDFNQTQPERGDNNLTR

SEQ ID NO: 18 - protein, 345 aa, synthetic construct
  REGION 1..345: note = Description of Artificial Sequence: Synthetic polypeptide
ANSFLFWNKYKDGDQCETSPCQNQGKCKDGLGEYTCTCLEGFEGKNCELFTRKLCSLDNGDCDQFCHEEQNSVVCSCARGYTLADNGKACIPTGPYPCGKQTLERRKRRKRIVGGQECKDGECPWQALLINEENEGFCGGTILSEFYILTAAHCLYQAKRFKVRVGDRNTEQEEGGEAVHEVEVVIKHNRFTKETYDFDIAVLRLKTPITFRMNVAPACLPERDWAESTLMTQKTGIVSGFGRTHEKGRQSTRLKMLEVPYVDRNSCKLSSSFIITQNMFCAGYDTKQEDACQGDAGGPHVTRFKDTYFVTGIVSWGEGCARKGKYGIYTKVTAFLKWIDRSMKT

SEQ ID NO: 19 - protein, 352 aa, synthetic construct
  REGION 1..352: note = Description of Artificial Sequence: Synthetic polypeptide
ANSFLFWNKYKDGDQCETSPCQNQGKCKDGLGEYTCTCLEGFEGKNCELFTRKLCSLDNGDCDQFCHEEQNSVVCSCARGYTLADNGKACIPTGPYPCGKQTLERRKRRKRIVGGQECKDGECPWQALLINEENEGFCGGTILSEFYILTAAHCLYQAKRFKVRVGDRNTEQEEGGEAVHEVEVVIKHNRFTKETYDFDIAVLRLKTPITFRMNVAPACLPERDWAESTLMTQKTGIVSGFGRTHEKGRQSTRLKMLEVPYVDRNSCKLSSSFIITQNMFCAGYDTKQEDACQGDAGGPHVTRFKDTYFVTGIVSWGEGCARKGKYGIYTKVTAFLKWIDRSMKTRGLPKAK

SEQ ID NO: 20 - protein, 350 aa, synthetic construct
  REGION 1..350: note = Description of Artificial Sequence: Synthetic polypeptide
ANSFLFWNKYKDGDQCETSPCQNQGKCKDGLGEYTCTCLEGFEGKNCELFTRKLCSLDNGDCDQFCHEEQNSVVCSCARGYTLADNGKACIPTGPYPCGKQTLERRKRRKRIVGGQECKDGECPWQALLINEENEGFCGGTILSEFYILTAAHCLYQAKRFKVRVGDRNTEQEEGGEAVHEVEVVIKHNRFTKETYDFDIAVLRLKTPITFRMNVAPACLPERDWAESTLMTQKTGIVSGFGRTHEKGRQSTRLKMLEVPYVDRNSCKLSSSFIITQNMFCAGYDTKQEDACQGDAGGPHVTRFKDTYFVTGIVSWGEGCARKGKYGIYTKVTAFLKWIDRSMKTRGLPK

SEQ ID NO: 21 - protein, 405 aa, synthetic construct
  REGION 1..405: note = Description of Artificial Sequence: Synthetic polypeptide
ANSFLFWNKYKDGDQCETSPCQNQGKCKDGLGEYTCTCLEGFEGKNCELFTRKLCSLDNGDCDQFCHEEQNSVVCSCARGYTLADNGKACIPTGPYPCGKQTLERRKRSVAQATSSSGEAPDSITWKPYDAADLDPTENPFDLLDFNQTQPERGDNNLTRRKRRKRIVGGQECKDGECPWQALLINEENEGFCGGTILSEFYILTAAHCLYQAKRFKVRVGDRNTEQEEGGEAVHEVEVVIKHNRFTKETYDFDIAVLRLKTPITFRMNVAPACLPERDWAESTLMTQKTGIVSGFGRTHEKGRQSTRLKMLEVPYVDRNSCKLSSSFIITQNMFCAGYDTKQEDACQGDAGGPHVTRFKDTYFVTGIVSWGEGCARKGKYGIYTKVTAFLKWIDRSMKTRGLPK

SEQ ID NO: 22 - protein, 409 aa, synthetic construct
  REGION 1..409: note = Description of Artificial Sequence: Synthetic polypeptide
DGDQCETSPCQNQGKCKDGLGEYTCTCLEGFEGKNCELFTRKLCSLDNGDCDQFCHEEQNSVVCSCARGYTLADNGKACIPTGPYPCGKQTLERRKRSVAQATSSSGEAPDSITWKPYDAADLDPTENPFDLLDFNQTQPERGDNNLTRRKRRKRIVGGQECKDGECPWQALLINEENEGFCGGTILSEFYILTAAHCLYQAKRFKVRVGDRNTEQEEGGEAVHEVEVVIKHNRFTKETYDFDIAVLRLKTPITFRMNVAPACLPERDWAESTLMTQKTGIVSGFGRTHEKGRQSTRLKMLEVPYVDRNSCKLSSSFIITQNMFCAGYDTKQEDACQGDAGGPHVTRFKDTYFVTGIVSWGEGCARKGKYGIYTKVTAFLKWIDRSMKTRGLPKAKSHAPEVITSSPLK

SEQ ID NO: 23 - protein, 394 aa, synthetic construct
  REGION 1..394: note = Description of Artificial Sequence: Synthetic polypeptide
DGDQCETSPCQNQGKCKDGLGEYTCTCLEGFEGKNCELFTRKLCSLDNGDCDQFCHEEQNSVVCSCARGYTLADNGKACIPTGPYPCGKQTLERRKRSVAQATSSSGEAPDSITWKPYDAADLDPTENPFDLLDFNQTQPERGDNNLTRRKRRKRIVGGQECKDGECPWQALLINEENEGFCGGTILSEFYILTAAHCLYQAKRFKVRVGDRNTEQEEGGEAVHEVEVVIKHNRFTKETYDFDIAVLRLKTPITFRMNVAPACLPERDWAESTLMTQKTGIVSGFGRTHEKGRQSTRLKMLEVPYVDRNSCKLSSSFIITQNMFCAGYDTKQEDACQGDAGGPHVTRFKDTYFVTGIVSWGEGCARKGKYGIYTKVTAFLKWIDRSMKTRGLPK

SEQ ID NO: 24 - protein, 391 aa, synthetic construct
  REGION 1..391: note = Description of Artificial Sequence: Synthetic polypeptide
DGDQCETSPCQNQGKCKDGLGEYTCTCLEGFEGKNCELFTRKLCSLDNGDCDQFCHEEQNSVVCSCARGYTLADNGKACIPTGPYPCGKQTLERSVAQATSSSGEAPDSITWKPYDAADLDPTENPFDLLDFNQTQPERGDNNLTRRKRRKRIVGGQECKDGECPWQALLINEENEGFCGGTILSEFYILTAAHCLYQAKRFKVRVGDRNTEQEEGGEAVHEVEVVIKHNRFTKETYDFDIAVLRLKTPITFRMNVAPACLPERDWAESTLMTQKTGIVSGFGRTHEKGRQSTRLKMLEVPYVDRNSCKLSSSFIITQNMFCAGYDTKQEDACQGDAGGPHVTRFKDTYFVTGIVSWGEGCARKGKYGIYTKVTAFLKWIDRSMKTRGLPK

SEQ ID NO: 25 - protein, 391 aa, synthetic construct
  REGION 1..391: note = Description of Artificial Sequence: Synthetic polypeptide
DGDQCETSPCQNQGKCKDGLGEYTCTCLEGFEGKNCELFTRKLCSLDNGDCDQFCHEEQNSVVCSCARGYTLADNGKACIPTGPYPCGKQTLERRKRRKRIVGGQECKDGECPWQALLINEENEGFCGGTILSEFYILTAAHCLYQAKRFKVRVGDRNTEQEEGGEAVHEVEVVIKHNRFTKETYDFDIAVLRLKTPITFRMNVAPACLPERDWAESTLMTQKTGIVSGFGRTHEKGRQSTRLKMLEVPYVDRNSCKLSSSFIITQNMFCAGYDTKQEDACQGDAGGPHVTRFKDTYFVTGIVSWGEGCARKGKYGIYTKVTAFLKWIDRSMKTRGLPKSVAQATSSSGEAPDSITWKPYDAADLDPTENPFDLLDFNQTQPERGDNNLTR

SEQ ID NO: 26 - protein, 422 aa, synthetic construct
  REGION 1..422: note = Description of Artificial Sequence: Synthetic polypeptide
DGDQCETSPCQNQGKCKDGLGEYTCTCLEGFEGKNCELFTRKLCSLDNGDCDQFCHEEQNSVVCSCARGYTLADNGKACIPTGPYPCGKQTLERRKRRKRIVGGQECKDGECPWQALLINEENEGFCGGTILSEFYILTAAHCLYQAKRFKVRVGDRNTEQEEGGEAVHEVEVVIKHNRFTKETYDFDIAVLRLKTPITFRMNVAPACLPERDWAESTLMTQKTGIVSGFGRTHEKGRQSTRLKMLEVPYVDRNSCKLSSSFIITQNMFCAGYDTKQEDACQGDAGGPHVTRFKDTYFVTGIVSWGEGCARKGKYGIYTKVTAFLKWIDRSMKTRGLPKSSGGSGGSGGSGGSGGSGGSGGSGGSGGSGSSVAQATSSSGEAPDSITWKPYDAADLDPTENPFDLLDFNQTQPERGDNNLTR

SEQ ID NO: 27 - protein, 950 aa, synthetic construct
  REGION 1..950: note = Description of Artificial Sequence: Synthetic polypeptide
DAHKSEVAHRFKDLGEENFKALVLIAFAQYLQQSPFEDHVKLVNEVTEFAKTCVADESAENCDKSLHTLFGDKLCTVATLRETYGEMADCCAKQEPERNECFLQHKDDNPNLPRLVRPEVDVMCTAFHDNEETFLKKYLYEIARRHPYFYAPELLFFAKRYKAAFTECCQAADKAACLLPKLDELRDEGKASSAKQRLKCASLQKFGERAFKAWAVARLSQRFPKAEFAEVSKLVTDLTKVHTECCHGDLLECADDRADLAKYICENQDSISSKLKECCEKPLLEKSHCIAEVENDEMPADLPSLAADFVESKDVCKNYAEAKDVFLGMFLYEYARRHPDYSVVLLLRLAKTYETTLEKCCAAADPHECYAKVFDEFKPLVEEPQNLIKQNCELFEQLGEYKFQNALLVRYTKKVPQVSTPTLVEVSRNLGKVGSKCCKHPEAKRMPCAEDYLSVVLNQLCVLHEKTPVSDRVTKCCTESLVNRRPCFSALEVDETYVPKEFNAETFTFHADICTLSEKERQIKKQTALVELVKHKPKATKEQLKAVMDDFAAFVEKCCKADDKETCFAEEGKKLVAASQAALGLANSFLFWNKYKDGDQCETSPCQNQGKCKDGLGEYTCTCLEGFEGKNCELFTRKLCSLDNGDCDQFCHEEQNSVVCSCARGYTLADNGKACIPTGPYPCGKQTLERRKRRKRIVGGQECKDGECPWQALLINEENEGFCGGTILSEFYILTAAHCLYQAKRFKVRVGDRNTEQEEGGEAVHEVEVVIKHNRFTKETYDFDIAVLRLKTPITFRMNVAPACLPERDWAESTLMTQKTGIVSGFGRTHEKGRQSTRLKMLEVPYVDRNSCKLSSSFIITQNMFCAGYDTKQEDACQGDAGGPHVTRFKDTYFVTGIVSWGEGCARKGKYGIYTKVTAFLKWIDRSMKTRGLPKAKSHAPEVITSSPLK

SEQ ID NO: 28 - protein, 935 aa, synthetic construct
  REGION 1..935: note = Description of Artificial Sequence: Synthetic polypeptide
ANSFLFWNKYKDGDQCETSPCQNQGKCKDGLGEYTCTCLEGFEGKNCELFTRKLCSLDNGDCDQFCHEEQNSVVCSCARGYTLADNGKACIPTGPYPCGKQTLERRKRRKRIVGGQECKDGECPWQALLINEENEGFCGGTILSEFYILTAAHCLYQAKRFKVRVGDRNTEQEEGGEAVHEVEVVIKHNRFTKETYDFDIAVLRLKTPITFRMNVAPACLPERDWAESTLMTQKTGIVSGFGRTHEKGRQSTRLKMLEVPYVDRNSCKLSSSFIITQNMFCAGYDTKQEDACQGDAGGPHVTRFKDTYFVTGIVSWGEGCARKGKYGIYTKVTAFLKWIDRSMKTRGLPKDAHKSEVAHRFKDLGEENFKALVLIAFAQYLQQSPFEDHVKLVNEVTEFAKTCVADESAENCDKSLHTLFGDKLCTVATLRETYGEMADCCAKQEPERNECFLQHKDDNPNLPRLVRPEVDVMCTAFHDNEETFLKKYLYEIARRHPYFYAPELLFFAKRYKAAFTECCQAADKAACLLPKLDELRDEGKASSAKQRLKCASLQKFGERAFKAWAVARLSQRFPKAEFAEVSKLVTDLTKVHTECCHGDLLECADDRADLAKYICENQDSISSKLKECCEKPLLEKSHCIAEVENDEMPADLPSLAADFVESKDVCKNYAEAKDVFLGMFLYEYARRHPDYSVVLLLRLAKTYETTLEKCCAAADPHECYAKVFDEFKPLVEEPQNLIKQNCELFEQLGEYKFQNALLVRYTKKVPQVSTPTLVEVSRNLGKVGSKCCKHPEAKRMPCAEDYLSVVLNQLCVLHEKTPVSDRVTKCCTESLVNRRPCFSALEVDETYVPKEFNAETFTFHADICTLSEKERQIKKQTALVELVKHKPKATKEQLKAVMDDFAAFVEKCCKADDKETCFAEEGKKLVAASQAALGL

SEQ ID NO: 29 - protein, 385 aa, synthetic construct
  REGION 1..385: note = Description of Artificial Sequence: Synthetic polypeptide
DGDQCETSPCQNQGKCKDGLGEYTCTCLEGFEGKNCELFTRKLCSLDNGDCDQFCHEEQNSVVCSCARGYTLADNGKACIPTGPYPCGKQTLERIVGGQECKDGECPWQALLINEENEGFCGGTILSEFYILTAAHCLYQAKRFKVRVGDRNTEQEEGGEAVHEVEVVIKHNRFTKETYDFDIAVLRLKTPITFRMNVAPACLPERDWAESTLMTQKTGIVSGFGRTHEKGRQSTRLKMLEVPYVDRNSCKLSSSFIITQNMFCAGYDTKQEDACQGDAGGPHVTRFKDTYFVTGIVSWGEGCARKGKYGIYTKVTAFLKWIDRSMKTRGLPKSVAQATSSSGEAPDSITWKPYDAADLDPTENPFDLLDFNQTQPERGDNNLTR

SEQ ID NO: 30 - protein, 416 aa, synthetic construct
  REGION 1..416: note = Description of Artificial Sequence: Synthetic polypeptide
DGDQCETSPCQNQGKCKDGLGEYTCTCLEGFEGKNCELFTRKLCSLDNGDCDQFCHEEQNSVVCSCARGYTLADNGKACIPTGPYPCGKQTLERIVGGQECKDGECPWQALLINEENEGFCGGTILSEFYILTAAHCLYQAKRFKVRVGDRNTEQEEGGEAVHEVEVVIKHNRFTKETYDFDIAVLRLKTPITFRMNVAPACLPERDWAESTLMTQKTGIVSGFGRTHEKGRQSTRLKMLEVPYVDRNSCKLSSSFIITQNMFCAGYDTKQEDACQGDAGGPHVTRFKDTYFVTGIVSWGEGCARKGKYGIYTKVTAFLKWIDRSMKTRGLPKSSGGSGGSGGSGGSGGSGGSGGSGGSGGSGSSVAQATSSSGEAPDSITWKPYDAADLDPTENPFDLLDFNQTQPERGDNNLTR

SEQ ID NO: 31 - protein, 35 aa, synthetic construct
  REGION 1..35: note = Description of Artificial Sequence: Synthetic polypeptide
AETVFPDVDYVNSTEAETILDNITQSTQSFNDFTR

SEQ ID NO: 32 - protein, 38 aa, synthetic construct
  REGION 1..38: note = Description of Artificial Sequence: Synthetic polypeptide
MSETSRTAFGGRRAVPPNNSNAAEDDLPTVELQGVVPR

SEQ ID NO: 33 - protein, 12 aa, synthetic construct
  REGION 1..12: note = Description of Artificial Sequence: Synthetic peptide
DTEDQEDQVDPR

SEQ ID NO: 34 - protein, 40 aa, Homo sapiens
MGRPLHLVLLSASLAGLLLLGESLFIRREQANNILARVTR

SEQ ID NO: 35 - protein, 24 aa, Homo sapiens
MAHVRGLQLPGCLALAALCSLVHS

SEQ ID NO: 36 - protein, 19 aa, Homo sapiens
MRLAVGALLVCAVLGLCLA

SEQ ID NO: 37 - protein, 43 aa, synthetic construct
  REGION 1..43: note = Description of Artificial Sequence: Synthetic polypeptide
MAHVRGLQLPGCLALAALCSLVHSQHVFLAPQQARSLLQRVRR

SEQ ID NO: 38 - protein, 20 aa, synthetic construct
  REGION 1..20: note = Description of Artificial Sequence: Synthetic peptide
RGLPKAKSHAPEVITSSPLK

SEQ ID NO: 39 - protein, 155 aa, synthetic construct
  REGION 1..155: note = Description of Artificial Sequence: Synthetic polypeptide
ANTFLEEVRKGNLERECVEETCSYEEAFEALESSTATDVFWAKYTACETARTPRDKLAACLEGNCAEGLGTNYRGHVNITRSGIECQLWRSRYPHKPEINSTTHPGADLQENFCRNPDSSTTGPWCYTTDPTVRRQECSIPVCGQDQVTVAMTPR

SEQ ID NO: 40 - protein, 129 aa, synthetic construct
  REGION 1..129: note = Description of Artificial Sequence: Synthetic polypeptide
SEGSSVNLSPPLEQCVPDRGQQYQGRLAVTTHGLPCLAWASAQAKALSKHQDFNSAVQLVENFCRNPDGDEEGVWCYVAGKPGDFGYCDLNYCEEAVEEETGDGLDEDSDRAIEGRTATSEYQTFFNPR

SEQ ID NO: 41 - protein, 471 aa, synthetic construct
  REGION 1..471: note = Description of Artificial Sequence: Synthetic polypeptide
ANSFLFWNKYKDGDQCETSPCQNQGKCKDGLGEYTCTCLEGFEGKNCELFTRKLCSLDNGDCDQFCHEEQNSVVCSCARGYTLADNGKACIPTGPYPCGKQTLERRKRSVAQATSSSGEAPDSITWKPYDAADLDPTENPFDLLDFNQTQPERGDNNLTRRKRRKRIVGGQECKDGECPWQALLINEENEGFCGGTILSEFYILTAAHCLYQAKRFKVRVGDRNTEQEEGGEAVHEVEVVIKHNRFTKETYDFDIAVLRLKTPITFRMNVAPACLPERDWAESTLMTQKTGIVSGFGRTHEKGRQSTRLKMLEVPYVDRNSCKLSSSFIITQNMFCAGYDTKQEDACQGDAGGPHVTRFKDTYFVTGIVSWGEGCARKGKYGIYTKVTAFLKWIDRSMKTRGLPKAKSHAPEVITSSPLKVAQATSSSGEAPDSITWKPYDAADLDPTENPFDLLDFNQTQPERGDNNLTR

SEQ ID NO: 42 - protein, 939 aa, synthetic construct
  REGION 1..939: note = Description of Artificial Sequence: Synthetic polypeptide
DAHKSEVAHRFKDLGEENFKALVLIAFAQYLQQSPFEDHVKLVNEVTEFAKTCVADESAENCDKSLHTLFGDKLCTVATLRETYGEMADCCAKQEPERNECFLQHKDDNPNLPRLVRPEVDVMCTAFHDNEETFLKKYLYEIARRHPYFYAPELLFFAKRYKAAFTECCQAADKAACLLPKLDELRDEGKASSAKQRLKCASLQKFGERAFKAWAVARLSQRFPKAEFAEVSKLVTDLTKVHTECCHGDLLECADDRADLAKYICENQDSISSKLKECCEKPLLEKSHCIAEVENDEMPADLPSLAADFVESKDVCKNYAEAKDVFLGMFLYEYARRHPDYSVVLLLRLAKTYETTLEKCCAAADPHECYAKVFDEFKPLVEEPQNLIKQNCELFEQLGEYKFQNALLVRYTKKVPQVSTPTLVEVSRNLGKVGSKCCKHPEAKRMPCAEDYLSVVLNQLCVLHEKTPVSDRVTKCCTESLVNRRPCFSALEVDETYVPKEFNAETFTFHADICTLSEKERQIKKQTALVELVKHKPKATKEQLKAVMDDFAAFVEKCCKADDKETCFAEEGKKLVAASQAALGLDGDQCETSPCQNQGKCKDGLGEYTCTCLEGFEGKNCELFTRKLCSLDNGDCDQFCHEEQNSVVCSCARGYTLADNGKACIPTGPYPCGKQTLERRKRRKRIVGGQECKDGECPWQALLINEENEGFCGGTILSEFYILTAAHCLYQAKRFKVRVGDRNTEQEEGGEAVHEVEVVIKHNRFTKETYDFDIAVLRLKTPITFRMNVAPACLPERDWAESTLMTQKTGIVSGFGRTHEKGRQSTRLKMLEVPYVDRNSCKLSSSFIITQNMFCAGYDTKQEDACQGDAGGPHVTRFKDTYFVTGIVSWGEGCARKGKYGIYTKVTAFLKWIDRSMKTRGLPKAKSHAPEVITSSPLK

SEQ ID NO: 43 - protein, 976 aa, synthetic construct
  REGION 1..976: note = Description of Artificial Sequence: Synthetic polypeptide
DAHKSEVAHRFKDLGEENFKALVLIAFAQYLQQSPFEDHVKLVNEVTEFAKTCVADESAENCDKSLHTLFGDKLCTVATLRETYGEMADCCAKQEPERNECFLQHKDDNPNLPRLVRPEVDVMCTAFHDNEETFLKKYLYEIARRHPYFYAPELLFFAKRYKAAFTECCQAADKAACLLPKLDELRDEGKASSAKQRLKCASLQKFGERAFKAWAVARLSQRFPKAEFAEVSKLVTDLTKVHTECCHGDLLECADDRADLAKYICENQDSISSKLKECCEKPLLEKSHCIAEVENDEMPADLPSLAADFVESKDVCKNYAEAKDVFLGMFLYEYARRHPDYSVVLLLRLAKTYETTLEKCCAAADPHECYAKVFDEFKPLVEEPQNLIKQNCELFEQLGEYKFQNALLVRYTKKVPQVSTPTLVEVSRNLGKVGSKCCKHPEAKRMPCAEDYLSVVLNQLCVLHEKTPVSDRVTKCCTESLVNRRPCFSALEVDETYVPKEFNAETFTFHADICTLSEKERQIKKQTALVELVKHKPKATKEQLKAVMDDFAAFVEKCCKADDKETCFAEEGKKLVAASQAALGLDGDQCETSPCQNQGKCKDGLGEYTCTCLEGFEGKNCELFTRKLCSLDNGDCDQFCHEEQNSVVCSCARGYTLADNGKACIPTGPYPCGKQTLERRKRRKRIVGGQECKDGECPWQALLINEENEGFCGGTILSEFYILTAAHCLYQAKRFKVRVGDRNTEQEEGGEAVHEVEVVIKHNRFTKETYDFDIAVLRLKTPITFRMNVAPACLPERDWAESTLMTQKTGIVSGFGRTHEKGRQSTRLKMLEVPYVDRNSCKLSSSFIITQNMFCAGYDTKQEDACQGDAGGPHVTRFKDTYFVTGIVSWGEGCARKGKYGIYTKVTAFLKWIDRSMKTRGLPKSVAQATSSSGEAPDSITWKPYDAADLDPTENPFDLLDFNQTQPERGDNNLTR

SEQ ID NO: 44 - protein, 51 aa, synthetic construct
  REGION 1..51: note = Description of Artificial Sequence: Synthetic polypeptide
VAQATSSSGEAPDSITWKPYDAADLDPTENPFDLLDFNQTQPERGDNNLTR

SEQ ID NO: 45 - protein, 20 aa, Homo sapiens
METDTLLLWVLLLWVPGSTG

SEQ ID NO: 46 - protein, 330 aa, Homo sapiens [sequence omitted]

SEQ ID NO: 47 - protein, 735 aa, synthetic construct
  REGION 1..735: note = Description of Artificial Sequence: Synthetic polypeptide
MGRPLHLVLLSASLAGLLLLGESLFIRREQANNILARVTRANSFLFWNKYKDGDQCETSPCQNQGKCKDGLGEYTCTCLEGFEGKNCELFTRKLCSLDNGDCDQFCHEEQNSVVCSCARGYTLADNGKACIPTGPYPCGKQTLERRKRRKRIVGGQECKDGECPWQALLINEENEGFCGGTILSEFYILTAAHCLYQAKRFKVRVGDRNTEQEEGGEAVHEVEVVIKHNRFTKETYDFDIAVLRLKTPITFRMNVAPACLPERDWAESTLMTQKTGIVSGFGRTHEKGRQSTRLKMLEVPYVDRNSCKLSSSFIITQNMFCAGYDTKQEDACQGDAGGPHVTRFKDTYFVTGIVSWGEGCARKGKYGIYTKVTAFLKWIDRSMKTRGLPKAKSHAPEVITSSPLKASTKGPSVFPLAPSSKSTSGGTAALGCLVKDYFPEPVTVSWNSGALTSGVHTFPAVLQSSGLYSLSSVVTVPSSSLGTQTYICNVNHKPSNTKVDKKVEPKSCDKTHTCPPCPAPELLGGPSVFLFPPKPKDTLMISRTPEVTCVVVDVSHEDPEVKFNWYVDGVEVHNAKTKPREEQYNSTYRVVSVLTVLHQDWLNGKEYKCKVSNKALPAPIEKTISKAKGQPREPQVYTLPPSRDELTKNQVSLTCLVKGFYPSDIAVEWESNGQPENNYKTTPPVLDSDGSFFLYSKLTVDKSRWQQGNVFSCSVMHEALHNHYTQKSLSLSPGK

SEQ ID NO: 48 - protein, 715 aa, synthetic construct
  REGION 1..715: note = Description of Artificial Sequence: Synthetic polypeptide
METDTLLLWVLLLWVPGSTGANSFLFWNKYKDGDQCETSPCQNQGKCKDGLGEYTCTCLEGFEGKNCELFTRKLCSLDNGDCDQFCHEEQNSVVCSCARGYTLADNGKACIPTGPYPCGKQTLERRKRRKRIVGGQECKDGECPWQALLINEENEGFCGGTILSEFYILTAAHCLYQAKRFKVRVGDRNTEQEEGGEAVHEVEVVIKHNRFTKETYDFDIAVLRLKTPITFRMNVAPACLPERDWAESTLMTQKTGIVSGFGRTHEKGRQSTRLKMLEVPYVDRNSCKLSSSFIITQNMFCAGYDTKQEDACQGDAGGPHVTRFKDTYFVTGIVSWGEGCARKGKYGIYTKVTAFLKWIDRSMKTRGLPKAKSHAPEVITSSPLKASTKGPSVFPLAPSSKSTSGGTAALGCLVKDYFPEPVTVSWNSGALTSGVHTFPAVLQSSGLYSLSSVVTVPSSSLGTQTYICNVNHKPSNTKVDKKVEPKSCDKTHTCPPCPAPELLGGPSVFLFPPKPKDTLMISRTPEVTCVVVDVSHEDPEVKFNWYVDGVEVHNAKTKPREEQYNSTYRVVSVLTVLHQDWLNGKEYKCKVSNKALPAPIEKTISKAKGQPREPQVYTLPPSRDELTKNQVSLTCLVKGFYPSDIAVEWESNGQPENNYKTTPPVLDSDGSFFLYSKLTVDKSRWQQGNVFSCSVMHEALHNHYTQKSLSLSPGK

SEQ ID NO: 49 - protein, 33 aa, synthetic construct
  REGION 1..33: note = Description of Artificial Sequence: Synthetic polypeptide
KSSGGSGGSGGSGGSGGSGGSGGSGGSGGSGSS